European Patent Application EP 4 455 292 A1, published October 30, 2024. Title: A METHOD FOR DETECTING ECTOINE. Applicant: Kaunas University of Technology. Application EP K158-101. The sequence listing filed with the application follows.

SEQUENCE LISTING (15 sequences)

SEQ ID NO: 1 - DNA, 1398 bp, Pseudomonas putida
  source 1..1398: mol_type = genomic DNA
atggaaaaatggcgggaagcggttgagcacgcccgtggcggcgagtccaagtacaagattcttgtccaagcgatcagctcggacatcgagcagcataagctggcggatgatcagcgcctgccacctcaacggcaggttgccgatgccttggggatcagtgtccaaaccgtgacaaacgcctacaaggaactcgagcgccaagggctagtaaggtgcgaagtgggtcgcgggagtttcgtttctcggcgaatgagtgaccgtgtagcaagctacattctcgatgctcccgagcgcgcactcgtcgatctatccaccgcccgaatcattcacaccccagagcatgacaggtactggcgagaaacatgcgccgagcttgctaatgaggtcgatcaaagctggatccgactgtgccgacctgtagcgggcttcgatgctcatcgtgatgccgcctgccattggcttgggcgtcttggattgccagggctggctcgagaagatgtgttgatcacaaatggggcggcccacgggctattcctggcgctggcctcccttgcaggccctgatgacctggtgctctgtgaaggcatgaccgatcacggtgtcattgggaactctcaagtcctcggcttcaatctgaaaggcctagacactgatcgtgacgggattgatcccgagcactttgaggacatctgcagcaacgagcgcgttacggccctggtatgcacgccgaaccttaataacccgaccagcgcgttgatgcccaatagccgcaggaaagagatagcctccatcgctcgtcgcttcggtgtccacattattgaggatgacgtctacggccccctgcttaaccaatacgaaggccctccaatcagctcatatgcccccgagctctcgttttactgcaccagcatgacgaagtcagttctgactgggctacgaatcgggttcctcaaagtacctaaacgactggcgctgcgaacagaaagcatccttcgcgtgacgagctggatggcagcccccatgcttgccgaggttgccgcacggtggattatggatgggagggccgacacattgatccaattgcagcgaaggctcctagagacacgccagaagctggtagcagacgagatggggcgctacctctattgccatcgccctcattcgttaaacgcttggctgaatgtgccagcacattgggatgtttccagcctggtgcgcacactacgacaacagcatattgcggttacgtcaccggagccgttcaccgttcggggggtgaccccagcacgcggcatccggctttgcatcggcgctgaaacgagtgaaagcgagctatcccaggccctgaaaaccatgcggatgacttttgaacaatacccaggagtccatgacttctga

SEQ ID NO: 2 - DNA, 16 bp, Pseudomonas putida
  source 1..16: mol_type = genomic DNA
attgccctagtacatt

SEQ ID NO: 3 - DNA, 44 bp, Pseudomonas putida
  source 1..44: mol_type = genomic DNA
attgccctagtacattcattatgacaatcagcggctcgtataat

SEQ ID NO: 4 - DNA, 43 bp, Pseudomonas putida
  source 1..43: mol_type = genomic DNA
attgccctagtacattcccttttaatcatccggctcgtataat

SEQ ID NO: 5 - DNA, 54 bp, Pseudomonas putida
  source 1..54: mol_type = genomic DNA
acgggtggcgattgccctagtacattcattatgacaatcagcggctcgtagact

SEQ ID NO: 6 - DNA, 54 bp, Pseudomonas putida
  source 1..54: mol_type = genomic DNA
acgccaccgctaacgcctagtacattcattatgacaatcagcggctcgtagact

SEQ ID NO: 7 - DNA, 44 bp, Pseudomonas putida
  source 1..44: mol_type = genomic DNA
attgcggatcaacattcattatgacaatcagcggctcgtagact

SEQ ID NO: 8 - DNA, 44 bp, Pseudomonas putida
  source 1..44: mol_type = genomic DNA
attgccctagttgtaagattatgacaatcagcggctcgtagact

SEQ ID NO: 9 - DNA, 44 bp, Pseudomonas putida
  source 1..44: mol_type = genomic DNA
attgccctagtacattctaatacacaatcagcggctcgtagact

SEQ ID NO: 10 - DNA, 44 bp, Pseudomonas putida
  source 1..44: mol_type = genomic DNA
attgccctagtacattcattatgtgttagagcggctcgtagact

SEQ ID NO: 11 - DNA, 44 bp, Pseudomonas putida
  source 1..44: mol_type = genomic DNA
attgccctagtacattcattatgacaatctcgccgtcgtagact

SEQ ID NO: 12 - DNA, 44 bp, Pseudomonas putida
  source 1..44: mol_type = genomic DNA
attgccctagtacattcattatgacaatcagcggcagcatcact

SEQ ID NO: 13 - DNA, 77 bp, Pseudomonas putida
  source 1..77: mol_type = genomic DNA
attgccctagtacattcattatgacaatcagcggctcgtagtgagacaaaaaaacaatcgttcggtggtctcatatg

SEQ ID NO: 14 - DNA, 77 bp, Pseudomonas putida
  source 1..77: mol_type = genomic DNA
attgccctagtacattcattatgacaatcagcggctcgtagactctgttttttacaatcgttcggtggtctcatatg

SEQ ID NO: 15 - DNA, 77 bp, Pseudomonas putida
  source 1..77: mol_type = genomic DNA
attgccctagtacattcattatgacaatcagcggctcgtagactctgaaaaaatgttaggttcggtggtctcatatg